European Patent Specification EP 3 874 067 B1, published April 3, 2024. Title: SELF-ASSEMBLING NUCLEIC ACID SURFACES FOR BIOSENSOR APPLICATIONS. Applicant: INSTITUT NATIONAL DE LA RECHERCHE SCIENTIFIQUE. The sequence listing filed with the application follows.

SEQUENCE LISTING (20 sequences)

SEQ ID NO: 1 - DNA, 17 bp, Artificial Sequence
  Nucleic Acid
  modified_base (17)..(17): Residue is thiolated
ggcgtgcgcgttccatg

SEQ ID NO: 2 - DNA, 37 bp, Artificial Sequence
  Nucleic Acid
aaacctgtcataacttactgtcctgatcggaaggatc

SEQ ID NO: 3 - DNA, 55 bp, Artificial Sequence
  Nucleic Acid
gtaagttatgacaggtttctagatctttgctcacgctgtcctgatcggaaggatc

SEQ ID NO: 4 - DNA, 55 bp, Artificial Sequence
  Nucleic Acid
gcgtgagcaaagatctagacatggaacgcgcacgcctgtcctgatcggaaggatc

SEQ ID NO: 5 - DNA, 55 bp, Artificial Sequence
  Nucleic Acid
ctgtagtgagttcgagacaaggaccattgcatgcgagatccttccgatcaggaca

SEQ ID NO: 6 - DNA, 55 bp, Artificial Sequence
  Nucleic Acid
tcgcatgcaatggtccttcaatgatatccctggatggatccttccgatcaggaca

SEQ ID NO: 7 - DNA, 55 bp, Artificial Sequence
  Nucleic Acid
catccagggatatagtgggtcgagaactcactacaggatccttccgatcaggaca

SEQ ID NO: 8 - DNA, 39 bp, Artificial Sequence
  Nucleic Acid
  modified_base (39)..(39): Residue is thiolated
ctctcaaagtattatgcaggacggcgtgcgcgttccatg

SEQ ID NO: 9 - DNA, 70 bp, Artificial Sequence
  Nucleic Acid
aaacctgtcataacttacctgagactagttggaagtgtggcatagctttcatgtcctgatcggaaggatc

SEQ ID NO: 10 - DNA, 110 bp, Artificial Sequence
  Nucleic Acid
ccacacttccaactagtctcaggtaagttatgacaggtttctagatctttgctcacgcatctagtcggtccacgtttggtcatagctttcatgtcctgatcggaaggatc

SEQ ID NO: 11 - DNA, 110 bp, Artificial Sequence
  Nucleic Acid
accaaacgtggaccgactagatgcgtgagcaaagatctagacatggaacgcgcacgccgtcctgcataatactttgagagcatagctttcatgtcctgatcggaaggatc

SEQ ID NO: 12 - DNA, 65 bp, Artificial Sequence
  Nucleic Acid
gttggcgcccgaccctcagactctgtagtgagttctatgtttttttttttttttttttttttttt

SEQ ID NO: 13 - DNA, 70 bp, Artificial Sequence
  Nucleic Acid
ccgagccattgcatgcgagatcggtagattgataggggatgatccttccgatcaggacatgaaagctatg

SEQ ID NO: 14 - DNA, 110 bp, Artificial Sequence
  Nucleic Acid
atcccctatcaatctaccgatctcgcatgcaatggctcggacagaatatccctggatgcaatagacggacagcttggtatgatccttccgatcaggacatgaaagctatg

SEQ ID NO: 15 - DNA, 110 bp, Artificial Sequence
  Nucleic Acid
ataccaagctgtccgtctattgcatccagggatattctgtacatagaactcactacagagtctgagggtcgggcgccaacgatccttccgatcaggacatgaaagctatg

SEQ ID NO: 16 - DNA, 64 bp, Artificial Sequence
  Nucleic Acid
cacaggctacggcacgtagagcatcaccatgatcctgtgaaaaaaaaaaaaaaaaaaaaaaaaa

SEQ ID NO: 17 - DNA, 57 bp, Artificial Sequence
  Nucleic Acid
ctgaacatccacactttagtaaacctgtcataacttactgtcctgatcggaaggatc

SEQ ID NO: 18 - DNA, 38 bp, Artificial Sequence
  Nucleic Acid
ggcgtgcgcgttccatgtctgaatcgatgcgcggcttc

SEQ ID NO: 19 - DNA, 57 bp, Artificial Sequence
  Nucleic Acid
actaaagtgtggatgttcagaaacctgtcataacttactgtcctgatcggaaggatc

SEQ ID NO: 20 - DNA, 38 bp, Artificial Sequence
  Nucleic Acid
ggcgtgcgcgttccatgtgaagccgcgcatcgattcag